European Patent Specification EP 3 986 555 B1, published May 6, 2026. Title: METHODS FOR TREATING NEOINTIMAL HYPERPLASIA USING F11R/JAM-A INHIBITORS. Applicant: The Research Foundation for the State University of New York. The sequence listing filed with the application follows.

SEQUENCE LISTING (17 sequences)

SEQ ID NO: 1 - protein, 13 aa, Artificial Sequence
  Laboratory synthesized sequence
  MISC_FEATURE (1)..(1): Xaa is Lys or D-Lys
  MISC_FEATURE (5)..(5): Xaa is Arg or D-Arg
  MOD_RES (13)..(13): OPTIONAL AMIDATION
XSVTXEDTGTYTC

SEQ ID NO: 2 - protein, 13 aa, Artificial Sequence
  Laboratory synthesized sequence
KSVTREDTGTYTC

SEQ ID NO: 3 - protein, 13 aa, Artificial Sequence
  Laboratory synthesized sequence
  MISC_FEATURE (1)..(1): Xaa is D-Lys
  MISC_FEATURE (5)..(5): Xaa is D-Arg
  MOD_RES (13)..(13): AMIDATION
XSVTXEDTGTYTC

SEQ ID NO: 4 - protein, 13 aa, Artificial Sequence
  Laboratory synthesized sequence
  MOD_RES (13)..(13): AMIDATION
KSVTREDTGTYTC

SEQ ID NO: 5 - protein, 13 aa, Artificial Sequence
  Laboratory synthesized sequence
  MISC_FEATURE (5)..(5): Xaa is D-Arg
  MOD_RES (13)..(13): AMIDATION
KSVTXEDTGTYTC

SEQ ID NO: 6 - protein, 13 aa, Artificial Sequence
  Laboratory synthesized sequence
  MISC_FEATURE (1)..(1): Xaa is R-Lys
  MOD_RES (13)..(13): AMIDATION
XSVTREDTGTYTX

SEQ ID NO: 7 - protein, 13 aa, Artificial Sequence
  Laboratory synthesized sequence
  MISC_FEATURE (5)..(5): Xaa is D-Arg
KSVTXEDTGTYTC

SEQ ID NO: 8 - protein, 13 aa, Artificial Sequence
  Laboratory synthesized sequence
  MISC_FEATURE (1)..(1): Xaa is D-Lys
XSVTREDTGTYTC

SEQ ID NO: 9 - protein, 13 aa, Artificial Sequence
  Laboratory synthesized sequence
  MISC_FEATURE (1)..(1): Xaa is D-Lys
  MISC_FEATURE (5)..(5): Xaa is D-Arg
XSVTXEDTGTYTC

SEQ ID NO: 10 - protein, 23 aa, Artificial Sequence
  Laboratory synthesized sequence
  MISC_FEATURE (12)..(12): Xaa is Arg or D-Arg
  MOD_RES (23)..(23): OPTIONAL AMIDATION
SVTVHSSEPEVXIPENNPVKLSC

SEQ ID NO: 11 - protein, 23 aa, Artificial Sequence
  Laboratory synthesized sequence
  misc_feature (12)..(12): Xaa can be any naturally occurring amino acid
SVTVHSSEPEVXIPENNPVKLSC

SEQ ID NO: 12 - protein, 23 aa, Artificial Sequence
  Laboratory synthesized sequence
  MOD_RES (23)..(23): AMIDATION
SVTVHSSEPEVRIPENNPVKLSC

SEQ ID NO: 13 - protein, 23 aa, Artificial Sequence
  Laboratory synthesized sequence
  MISC_FEATURE (12)..(12): Xaa is D-Arg
SVTVHSSEPEVXIPENNPVKLSC

SEQ ID NO: 14 - protein, 23 aa, Artificial Sequence
  Laboratory synthesized sequence
  MISC_FEATURE (12)..(12): Xaa is D-Arg
  MOD_RES (23)..(23): AMIDATION
SVTVHSSEPEVXIPENNPVKLSC

SEQ ID NO: 15 - protein, 14 aa, Artificial Sequence
  Laboratory synthesized sequence
  MISC_FEATURE (7)..(7): Xaa is Arg or D-Arg
SSEPEVXIPENNPV

SEQ ID NO: 16 - protein, 14 aa, Artificial Sequence
  Laboratory synthesized sequence
SSEPEVRIPENNPV

SEQ ID NO: 17 - protein, 14 aa, Artificial Sequence
  Laboratory synthesized sequence
  MISC_FEATURE (7)..(7): Xaa is D-Arg
SSEPEVXIPENNPV